European Patent Specification EP 3 746 088 B1, published July 10, 2024. Title: COMPOSITIONS AND METHODS FOR INDUCING TRIPARTITE MOTIF-CONTAINING PROTEIN 16 (TRIM16) SIGNALING. Applicant: University of Washington Gale, M.J. The sequence listing filed with the application follows.

SEQUENCE LISTING (91 sequences)

SEQ ID NO: 1 - protein, 564 aa, Homo sapiens [sequence omitted]

SEQ ID NO: 2 - RNA, 105 nt, Artificial Sequence
  Synthetic RNA
ggccauccuguuuuuuucccuuuuuuuuuuucuuuuuuuuuuuuuuuuuuuuuuuuuuuuuuuuuucuccuuuuuuuuuccucuuuuuuuccuuuucuuuccuuu

SEQ ID NO: 3 - RNA, 107 nt, Artificial Sequence
  Synthetic RNA
acuguuccuuuuuuuuuuuuuuuuuuuuuuuuuuuuuuuuuuuuuuuuuuucuuuuuuuuuuuuuucccucuuucuucccuucucaucuuauucuacuuucuuucuu

SEQ ID NO: 4 - RNA, 131 nt, Artificial Sequence
  Synthetic RNA
ggccauccuguuuuuuucccuuuuuuuuuuucuuuuuuuuuuuuuuuuuuuuuuuuuuuuuuuuuucuccuuuuuuuuuccucuuuuuuuccuuuucuuuccuuucccccccccccccccccccccccccc

SEQ ID NO: 5 - RNA, 105 nt, Artificial Sequence
  Synthetic RNA
ggccauccuguuuuuuucccuuuuuuuuuuucuuuuuuuuuuuuuuuuuuuuuuuuuuuuuuuuuucuccuuuuuuuuucccccccccccccccccccccccccc

SEQ ID NO: 6 - RNA, 105 nt, Artificial Sequence
  Synthetic RNA
ggccauccuguuuuuuucccuuuuuuuuuuucuuuuuuuuuuuuuuuuuuuuuuuuuuuuuuuuuuuuccuuuuuuuuuccucuuuuuuuccuuuucuuuccuuu

SEQ ID NO: 7 - RNA, 105 nt, Artificial Sequence
  Synthetic RNA
uuuuuuuuuuuuuuuuuuuuuuuuuuuuuuuuuuuuuuuuuuuuuuuuuuuuuuuuuuuuuuuuuuuuuuuuuuuuuuuuuuuuuuuuuuuuuuuuuuuuuuuuu

SEQ ID NO: 8 - RNA, 105 nt, Artificial Sequence
  Synthetic RNA
ggccauccuguuuuuuucccuuuuuuuuuuucuuuuuuuucuccuuuuuuuuuccucuuuuuuuccuuuucuuuccuuucccccccccccccccccccccccccc

SEQ ID NO: 9 - RNA, 105 nt, Artificial Sequence
  Synthetic RNA
ggccauccuguuuuuuucccuuuuuuuuuuucuuuuuuuuuuuuuuuuucuccuuuuuuuuuccucuuuuuuuccuuuucuuuccuuuccccccccccccccccc

SEQ ID NO: 10 - RNA, 62 nt, Artificial Sequence
  Synthetic RNA
ggccauccuguuuuuuuuuuuuuuuuuuuuuuuuuuuuuuuuuucuccuuuuuuuuuccucu

SEQ ID NO: 11 - RNA, 62 nt, Artificial Sequence
  Synthetic RNA
ccccccccccuuuuuuuuuuuuuuuuuuuuuuuuuuuuuuuuuucuccuuuuuuuuuccucu

SEQ ID NO: 12 - RNA, 62 nt, Artificial Sequence
  Synthetic RNA
ggccauccuguuuuuuuuuuuuuuuuuuuuuuuuuuuuuuuuuucccccccccccccccccc

SEQ ID NO: 13 - RNA, 62 nt, Artificial Sequence
  Synthetic RNA
uuuuuuuuuuuuuuuuuuuuuuuuuuuuuuuuuuuuuuuuuuuuuuuuuuuuuuuuuuuuuu

SEQ ID NO: 14 - RNA, 62 nt, Artificial Sequence
  Synthetic RNA
uuuuuuuuuuuuuuuuuuuuuuuuuuuuuuuuuuuuuuuuuuuucuuuuuuuuuuuuuuuuu

SEQ ID NO: 15 - RNA, 62 nt, Artificial Sequence
  Synthetic RNA
uuccuuccuuuuuuuuuuuuuuuuuuuuuuuuuuuuuuuuuuuucuccuuuuuuuuuccucu

SEQ ID NO: 16 - RNA, 62 nt, Artificial Sequence
  Synthetic RNA
uuuuuuuuuguuuuuuuuuuuuuuuuuuuuuuuuuuuuuuuuuucuccuuuuuuuuuccucu

SEQ ID NO: 17 - RNA, 62 nt, Artificial Sequence; identical to SEQ ID NO: 16
  Synthetic RNA

SEQ ID NO: 18 - RNA, 62 nt, Artificial Sequence
  Synthetic RNA
gguuuuccuuuuuuuuuuuuuuuuuuuuuuuuuuuuuuuuuuuucuuuuuuuuuuuuuuuuu

SEQ ID NO: 19 - RNA, 62 nt, Artificial Sequence
  Synthetic RNA
ggccauccuguuuuuuuuuucuuuuuuuuuucuuuuuuuuuucucuccuuuuuuuuuccucu

SEQ ID NO: 20 - RNA, 62 nt, Artificial Sequence
  Synthetic RNA
ggccauccuguuuuuuuuuuuuuuucuuuuuuuuuuuuuuucuucuccuuuuuuuuuccucu

SEQ ID NO: 21 - RNA, 62 nt, Artificial Sequence
  Synthetic RNA
ggccauccuguuuuuuuuuucccuuuuuuuuuucccuuuuuuuucuccuuuuuuuuuccucu

SEQ ID NO: 22 - RNA, 62 nt, Artificial Sequence
  Synthetic RNA
ggccauccuguuuuuuuuuuuuuuuuuuccccccuuuuuuuuuucuccuuuuuuuuuccucu

SEQ ID NO: 23 - RNA, 105 nt, Artificial Sequence; identical to SEQ ID NO: 2
  Synthetic RNA

SEQ ID NO: 24 - RNA, 35 nt, Artificial Sequence
  Synthetic RNA
ggccauucuuuuuuuuuuuuuuuucuuucuucuuu

SEQ ID NO: 25 - RNA, 116 nt, Artificial Sequence
  Synthetic RNA
ggccauucccuuuuuuuuuuuuuuuuuuuuuuuuuuuuuuuuuuuuuuuuuuuuuuuuuuuuuuuuuuuuuuuuuuuuuuuuuuuuuuuuucucuucuuuucuuuauuccuucuuu

SEQ ID NO: 26 - RNA, 101 nt, Artificial Sequence
  Synthetic RNA
ggccguuccuuuuuuuuuuuuuuuuuuuuuuuuuuuuuuuuuuuuuuuuuuuuuuuuuuuuuuuuuuuuuuuucuuuuccccuuuuuuauuuuucuuucuu

SEQ ID NO: 27 - RNA, 105 nt, Artificial Sequence
  Synthetic RNA
ggccauccuguuuuuuuguuuuuucuuuuuuuuuuuuuuuuuuuuuuuuuuuuuuuuuuuuuuuuuuucuuuuuuucccuuuuuuuuauuuuauuuucuuuuggu

SEQ ID NO: 28 - RNA, 131 nt, Artificial Sequence
  Synthetic RNA
ggccaucccccuuuuuuuuuuuuuuuuuuuuuuuuuuuuuuuuuuuuuuuuuuuuuuuuuuuuuuuuuuuuuuuuuuuuuuuuuuuuuuuuuuuuuuuuuuuuuuuuccucuuuuuuuccuuuucuucuuu

SEQ ID NO: 29 - RNA, 116 nt, Artificial Sequence
  Synthetic RNA
ggccguucuguuuuuuuuuuuuuuuuuuuuuuuuuuuuuuuuuuuuuuuuuuuuuuuuuuuuuuuuuuuuuuuuuuuuuuuuuuuuuuuuuuuuuccuuuuuuuuauuccucuucu

SEQ ID NO: 30 - RNA, 123 nt, Artificial Sequence
  Synthetic RNA
ggccauccccuuuguuuuuuuuuuuuuuuuuuuuuuuuuuuuuuuuuuuuuuuuuuuuuuuuuuuuuuuuuuuuuuuuuuuuuuuuuuuuuuuuuuuuuuuuuuuuuuauuucuccuucuuuu

SEQ ID NO: 31 - RNA, 87 nt, Artificial Sequence
  Synthetic RNA
ggccauuccuuuuuuuuuuuuuuuuuuuuuuuuucuuuuuuuuuccuuuuuuuuuuuuuuuuuuuuuuuuccuuuucuuucuucuuu

SEQ ID NO: 32 - RNA, 87 nt, Artificial Sequence; identical to SEQ ID NO: 31
  Synthetic RNA

SEQ ID NO: 33 - RNA, 96 nt, Artificial Sequence
  Synthetic RNA
agccauuuccuguuuuuuuuuuuuuuuuuuuuuuuuuuuucuuuuuuuuuuucuuuccuuuccuucuuuuuuuccuuucuuuuucccuucuuuaau

SEQ ID NO: 34 - RNA, 101 nt, Artificial Sequence
  Synthetic RNA
ggccauuuccuguuuuuuuuuuuuuuugguuuuuuuuuuuuuuuuuuuuuuuuuuuuuuuuuuuuuuuccuuuccuucuuuuuuuuuuuuucccucuuuau

SEQ ID NO: 35 - RNA, 87 nt, Artificial Sequence
  Synthetic RNA
ggccauuuccuguuuuuuuuuuuuuuuuuuuuuuuuuuuuuuuuuucuuuuccuucuuuuucccuuuuucuuucuuccuucuuuaau

SEQ ID NO: 36 - RNA, 100 nt, Artificial Sequence
  Synthetic RNA
ggccauccuguguuuuuuuuuuuuuuuuuuuuuuuuuuuuuuuuuuuuuuuuuuuuuuuuuuuuuuuuuuuuuuuuuuuuuuuuuuuauuuccuuuucuu

SEQ ID NO: 37 - RNA, 109 nt, Artificial Sequence
  Synthetic RNA
ggccaaccuguuuuuuuuuuuuuuuuuuuuuuuuuuccuuuuuuuuuuuuuuuuuuuuuuuuuuuuuuuuuuccuuuuuuucuuuuuuuuuuuuuuuuuccuuccuuuu

SEQ ID NO: 38 - RNA, 34 nt, Artificial Sequence
  Synthetic RNA
ggccauccuguuuuuuuuuuuuuuuucuuucuuu

SEQ ID NO: 39 - RNA, 74 nt, Artificial Sequence
  Synthetic RNA
ggccauuuuuccuuuuuuuuuuuuuuuuuuuuuuucuuuuuuuuuuccuuuuuuucuuuuuuuuucuuuucuuu

SEQ ID NO: 40 - RNA, 81 nt, Artificial Sequence
  Synthetic RNA
ggccauucuuuuuuuuuuuuuuuuuuuuuuuuuuuuuuuuuuucguuucuuuuucuucuuuuuguuuucucuucuccuuuu

SEQ ID NO: 41 - RNA, 107 nt, Artificial Sequence
  Synthetic RNA
ggccauuccccuuuuuuuuuuuuuuccgcuuuuuuuuuuuuuuuuuuuuuuuuuuuuuuuuucuuuuuuuuuccuuuuuuuuuuuuuuuuuuuuuuuuuuucuuuuu

SEQ ID NO: 42 - RNA, 109 nt, Artificial Sequence
  Synthetic RNA
ggccaucccccuuuuuuuuuuuuuccgcuuuuuuuuuuuuuuuuuuuuucuuuuuuuuuuucuuuuuuuuuuccuuuuuuuuuuuuuuuuuuuuuuuucuuuucuuuuu

SEQ ID NO: 43 - RNA, 35 nt, Artificial Sequence; identical to SEQ ID NO: 24
  Synthetic RNA

SEQ ID NO: 44 - RNA, 48 nt, Artificial Sequence
  Synthetic RNA
ggccauccccuucuuuuuuuuuuuuuuuuuuuuuuccuuuucuucuuu

SEQ ID NO: 45 - RNA, 100 nt, Artificial Sequence
  Synthetic RNA
ggccauccuguuuuuuucccuuuuuuuuuuucuuuuuuuuuuuuuuuuuuuuuuuuuuuuucuccuuuuuuuuuccucuuuuuuuccuuuucuuuccuuu

SEQ ID NO: 46 - RNA, 112 nt, Artificial Sequence
  Synthetic RNA
ggccguccuguuuuuuuuuuuuuuuuuuuccuuuuuuuuuuuuuuuuuuuuuuuuuuuuuuuuuuuuuuuuuuuuuuuuuuuuuuuuuuuuuuuuuuucuucuuucuuucuu

SEQ ID NO: 47 - RNA, 145 nt, Artificial Sequence
  Synthetic RNA
ggccauuuccuguuuuuuuuuuuuuuuuuuuuuuuuuuuuuuuuuuuuuuuuuuuuuuuuuuuuucuuuuuuuuuuuuuuuuuccuuuuuuuuuuuuuuuuuuuucuuuccuucuuuuuuccuuucuuuuccuuccuucuuuaau

SEQ ID NO: 48 - RNA, 95 nt, Artificial Sequence
  Synthetic RNA
ggccauuccuguuuuuuuuuuuuuuuucuuuuguuuuuuuuguuuuuuuuuuuuuuuuuccuuucuuuuuuuuuuuuuuuccuuucuucuuuaau

SEQ ID NO: 49 - RNA, 72 nt, Artificial Sequence
  Synthetic RNA
ggccauuuccuguuuuuuuuuuuuuuuuuuuucuuuccuucuuuuuuccuuucuuuuccuuccuucuuuaau

SEQ ID NO: 50 - RNA, 87 nt, Artificial Sequence; identical to SEQ ID NO: 35
  Synthetic RNA

SEQ ID NO: 51 - RNA, 143 nt, Artificial Sequence
  Synthetic RNA
ggccauuuccuguuuuuuuuuuuuuuuuuuuuuuuuuuuuuuuuuuuuuuuuuuuuuuuuuuucuuuuuuuuuuuuuuuuuccuuuuuuuuuuuuuuuuuuuucuuuccuucuuuuuuccuuucuuuuccuuccuucuuuaau

SEQ ID NO: 52 - RNA, 108 nt, Artificial Sequence
  Synthetic RNA
ggccauuuccuguuuuuuuuuuuuuucccuuuuuuuuuuuuuuuuuuuuuuuuuuuuuuuuuuuuucuuuccuucuuuuuuuuccuuucuuuuccuuccuucuuuaau

SEQ ID NO: 53 - RNA, 82 nt, Artificial Sequence
  Synthetic RNA
ggcauccuguuuuuuuuuuuuuuuuuuuuuuuuuuuuuuuuuuuuuuuuuuuuuuuuuuuuuuuuuuuuuuuucuuuucuuu

SEQ ID NO: 54 - RNA, 130 nt, Artificial Sequence
  Synthetic RNA
acacuccauuucuuuuuuuguuuuuuuuuuuuuuuuuuuuuuuuuuuuuuuuuuuuuuuuuuuuuuuuuuuuuuuuuuuuuuuuuuucuuuuucuuuccuuucuuuucugacuucuaauuuuccuucuua

SEQ ID NO: 55 - RNA, 129 nt, Artificial Sequence
  Synthetic RNA
guccuucuguuuuuuuuuuuuuuuuuuuuuuuuuuuuuuuuuuuuuuuuuuuuuuuuuuuuuuuuuuuuuuuuuuuuuuuuuuuuuuccuuacccuuuccuucuuuucuuccuuuuuuuuccuuacuuu

SEQ ID NO: 56 - RNA, 57 nt, Artificial Sequence
  Synthetic RNA
ggguccccuuguuuuuuuuuuuucuuuccuucuuuccuuuccuaaucuuucuuucuu

SEQ ID NO: 57 - RNA, 96 nt, Artificial Sequence; identical to SEQ ID NO: 33
  Synthetic RNA

SEQ ID NO: 58 - RNA, 115 nt, Artificial Sequence
  Synthetic RNA
ggccauuuccuguuuuuuuuuuuuuuuguuuuuuuuuuuuuuuuuuuuuuuuuuuuuuuuuuuuuuuuuuuuuuuuuuuuuuuccuuuccuuuuuuuuuuuuuuucccuuuuuau

SEQ ID NO: 59 - RNA, 107 nt, Artificial Sequence
  Synthetic RNA
ggccauccuguuuuuuuuuuuuuuuuuuuuuucuuuuuuuuuuuuuuuuucuuuuuuuuucuucuuuuucuuuccuuuuuuuuuuuuuuuuuuuuuuuucuucuuuc

SEQ ID NO: 60 - RNA, 96 nt, Artificial Sequence
  Synthetic RNA
ggccauuuccuguuuuuuuuuuuuuuuuuuuuuuuuuuuuuuuuuuuuuuuuuuuuuucuuuuucccucuuuuucuucucuuuuuccuucuuuaau

SEQ ID NO: 61 - RNA, 111 nt, Artificial Sequence
  Synthetic RNA
gcuaacuguuccuuuuuuuuuuuuuuuuuuuuuuuuuuuuuuuuuuuuuuuuuuucuuuuuuuuuuuuuucccucuuucuucccuucucaucuuauucuacuuucuuucuu

SEQ ID NO: 62 - RNA, 107 nt, Artificial Sequence
  Synthetic RNA
gcuaacuguuccuuuuuuuuuuuuuuuuuuuuuuuuuuuuuuuuuuuuuucuuuuuuuuuuuuuuucccucuuucuucccuucucaucuuauucuacuuucuuucuu

SEQ ID NO: 63 - RNA, 92 nt, Artificial Sequence
  Synthetic RNA
gcuaacuguuccuuuuuuuuuuucuuuuuuuuuuuuuuuuuuuuuuuuuuuccuucuuucuuucuuucuuaccuuacuuuacuuucuuuucu

SEQ ID NO: 64 - RNA, 111 nt, Artificial Sequence
  Synthetic RNA
gcuaacaguuucucuuuuuuuuuuuuuccuuuuuuauuuuuauuuuuuuuuuuuuuuuuuuuuuuuuauuuucuuuuccuuucuuucucaccuuacauuacuuucuuucuu

SEQ ID NO: 65 - RNA, 77 nt, Artificial Sequence
  Synthetic RNA
gcuaauuuccuuauuguuuuuuuuuuuuuuuuuuucuuuccauuuccuuccuucuuacuucacuuuaccuucuuucu

SEQ ID NO: 66 - RNA, 124 nt, Artificial Sequence
  Synthetic RNA
gcuaacuguuuuuuuuuuuuuuuuuuuuuuuuuuuuuuuuuuuuuuuuuuuuuuuuuuuuuuuuuuuuuuuuuuuuuuuuuuuuuccuuuccuuucuuucuuaccuuacuuuacauucuuuucu

SEQ ID NO: 67 - RNA, 119 nt, Artificial Sequence
  Synthetic RNA
gcuaacuguuccuuuuuuuuuuuuuuuuuuuuuuuuuuuuuuuuuuuuuuuuuuuuuuuuuuuuuuuuuuuuuuuuuuuuuucuuuccuuccuuucucaccuucuuuuacuucuuuccu

SEQ ID NO: 68 - RNA, 93 nt, Artificial Sequence
  Synthetic RNA
gcuaacuguuuuuuuuuuuuuuuuuuuuuuuuuuuuuuuuuuuuuuuuuuuuucuuuucuuuccuuuccuucuuacucuacuuuacuuuuucu

SEQ ID NO: 69 - RNA, 129 nt, Artificial Sequence
  Synthetic RNA
gcuaacuguucuuuuuuuuuuuuuuuuuuuuuuuuuuuuuuuuuuuuuuuuuuuuuuuuuuuuuuuuuuuuuuuuuuuuuuuuuuuuuucuuuuccuucuucuuucuuaccuuauuuuccuucuuucuu

SEQ ID NO: 70 - RNA, 86 nt, Artificial Sequence
  Synthetic RNA
gcuaacuguuuuuuuuuuuuuuuuuuuuuuuuuuuuuucuuuuuuuuucuuuucuuuccuucuuaccuuacuuuacuuucuuuucu

SEQ ID NO: 71 - RNA, 133 nt, Artificial Sequence
  Synthetic RNA
gcuaacuguuuuuuuuuuuuuuuuuuuuuuuuuuuuuuuuuuuuuuuuuuuuuuuuuuuuuuuuuuuuuuuuuuuuuuuuuuuuuuuuuccuuuuuccuuuuccuucucuuuuuaccuuacuuuacuuuucuu

SEQ ID NO: 72 - RNA, 144 nt, Artificial Sequence
  Synthetic RNA
gcuaacugucccuuuuuuuuuuuuuuuuuuuuuuuuuuuuuuuuuuuuuuuuuuuuuuuuuuuuuuuuuuuuuuuuuuuuuuuuuuuuuuuuuuuucuuuuuuucucuuuuccuucuuucuuaccuuauuuuacuuucuuuccu

SEQ ID NO: 73 - RNA, 119 nt, Artificial Sequence
  Synthetic RNA
gcuaacugucccuuuuuuuuuguuuuuuuuuuuuuuuuuuuuuuuuuuuuuucuuuuuuuuuuuuuuuuuuguuucuuuuccuucucauuuccuucuuaucuuaauuacuuccuuuccu

SEQ ID NO: 74 - RNA, 88 nt, Artificial Sequence
  Synthetic RNA
gcuaacuguuuuuuuuuuuuuuuuuuuuuuuuuuuuuuuuuuuuuuuccuucuuccuuuccuucuuaccuuacuuuauuuucuuuccu

SEQ ID NO: 75 - RNA, 101 nt, Artificial Sequence
  Synthetic RNA
gcuaacuguuuuuuuuuuuuuuuuuuuuuuuuuuuuuuuuuuuuuuuuuuuuuuuuuuuuuucuuucuuuucuuuucucaccuuacuuuacuuccuuucuu

SEQ ID NO: 76 - RNA, 86 nt, Artificial Sequence
  Synthetic RNA
gcuaguuuucuuuuuuuuuuuuuuuuuuuuuuuuguuuuuuuuuuuuuuccucuuuuuccguauuuuuuuuuuuuccucuuuucuu

SEQ ID NO: 77 - RNA, 105 nt, Artificial Sequence; identical to SEQ ID NO: 2
  Synthetic RNA

SEQ ID NO: 78 - RNA, 79 nt, Artificial Sequence
  Synthetic RNA
ccauuuuucuuuuuuuuuuuuuguuuguuuuuuuuuuuuuuuucuuuccuucuuuccugacuuuuaauuuuccuucuua

SEQ ID NO: 79 - RNA, 116 nt, Artificial Sequence
  Synthetic RNA
ccauuuuucuuuuuuuuuuuuuuuuuuuuuuuuuuuuuuuuuuuuuuuuuuuuuuuuuguuuguuuuuuuuuuuuuuuuucuuuccuucuuuccugacuuuuaauuuuccuucuua

SEQ ID NO: 80 - RNA, 84 nt, Artificial Sequence
  Synthetic RNA
ggccauuuccuguuuuuuuuuuuuuuuuuuuuuuuuuuuuuuuuuacccuuuuuucucuuuuuuuuuuuuccuucuucuuuaau

SEQ ID NO: 81 - RNA, 74 nt, Artificial Sequence
  Synthetic RNA
ggccauuuccuguuuuuuuuuuuuuuuuuuacccuuuuuucucuuuuuuuuuuuuuuuuuccuucuucuuuaau

SEQ ID NO: 82 - RNA, 38 nt, Artificial Sequence
  Synthetic RNA
ggccauuuucuguuuuuuuuuuuuuuauuuucuuuaau

SEQ ID NO: 83 - RNA, 53 nt, Artificial Sequence
  Synthetic RNA
ggccauuuucuuuuuuuuuucucuuuuuuuuuuuuuuuuuuauuuucuuuaau

SEQ ID NO: 84 - RNA, 82 nt, Artificial Sequence
  Synthetic RNA
ggccauuuucuguuuuuuuuuuuuuuuuuuuuccuuuuuuuuuuuuccucuuuuuuuuuuuuuuuuuuuuauuuucuuuaau

SEQ ID NO: 85 - RNA, 82 nt, Artificial Sequence
  Synthetic RNA
ggccauuuucuguuuuuuuuuuuucuuuuuuuuuuuuuuuuuccuuuuuuuuucucuuuuuuuuuuuuuuauuuucuuuaau

SEQ ID NO: 86 - RNA, 85 nt, Artificial Sequence
  Synthetic RNA
ggccauccuguuuuuuuuuuuuuuuuuuuuuuuuguuuuuuuuuuuuuuuuucuuuuuccuuuuuuuuuuuuuauuuucuucuuu

SEQ ID NO: 87 - RNA, 59 nt, Artificial Sequence
  Synthetic RNA
gguccuaaguuuuuuuuuuuuucuuccuuccuucuuuccuuuucuaauuuuccuucuuu

SEQ ID NO: 88 - RNA, 62 nt, Artificial Sequence
  Synthetic RNA
gguccuaaguuguuuuuuuuuuuuuuuccuuccuucuuucccuuuucuaauuuuccuucuuu

SEQ ID NO: 89 - RNA, 74 nt, Artificial Sequence
  Synthetic RNA
gguccuaaguuguuuuuuuuuuuuuuuuuuuuuuuccuuuccuuccuucuuuccuuuucuaauuuuccuucuuu

SEQ ID NO: 90 - RNA, 95 nt, Artificial Sequence
  Synthetic RNA
ggccauuucuguuuuuuuuuuuuuuuuuuuuuuuuuuuuuuuuuuuuuuuuuguuuccuucuuuuuccuuuucuuuuuuuuuuucucccuuuaau

SEQ ID NO: 91 - RNA, 70 nt, Artificial Sequence
  Synthetic RNA
ggccauuucuguuuuuuuuuuuuuuguuuccuucuuuuuccuuuucuuuuuuuuuuuuucucccuuuaau